European Patent Application EP 4 407 045 A1, published July 31, 2024. Title: NON-INVASIVE METHOD FOR THE DIAGNOSIS OF EOSINOPHILIC ESOPHAGITIS. Applicant: Universidad del Pais Vasco/Euskal Herriko Unibertsitatea (UPV/EHU). The sequence listing filed with the application follows.

SEQUENCE LISTING (27 sequences)

SEQ ID NO: 1 - DNA, 4602 bp, Homo sapiens
  source 1..4602: mol_type = other DNA; note = CDH26 cDNA ENST00000348616.9
agccagtcttttgtgtacgtgcaggaccatggtggctttagtttctaccccacccttcctaggaactctacttgtggcaaacgtatgttcaagcttacaagtcagcccaccccactctgataaatgcaagaaaagctgaaaagggaggagcaagatgggatgaaagcatctgggccaaagtgacctgaaaacctttagagaagaagctgctggctgagaaggaggtgtgtggctccggtgagaccaccagcttggaggactggtcatcagctgcacgttctgggtctgtcttgggtattcccatatggccatgagatccgggaggcacccctcgctgctgctgcttctagtgctgctgctgtggctgctgcaggtcagtatcattgacagtgttcaacaggaaacagatgatcttactaagcaaacaaaggaaaagatctaccagcctctacggcgatccaagagaagatgggttatcaccaccttggagctggaggaggaagacccgggaccctttcccaaactcattggtgagctgttcaataatatgtcttataacatgtcactaatgtatctaatcagtggacctggtgtggatgaatatccagagattggtttgttttctctagaagatcatgagaacggaaggatatatgttcaccgccctgtcgatcgagaaatgacaccatctttcacggtttattttgatgttgtggagcgctcaacaggaaaaattgtggatacatccttgattttcaacattaggatcagtgatgtgaatgatcatgcaccccagtttccagagaaggaatttaacatcactgtgcaagaaaaccaatctgcagggcaacctatttttcagatgttagcagtcgatttggatgaagaaaacactccaaattctcaagtcctttacttcctcatttctcaaacaccattactgaaagaaagtggtttccgggttgatcgccttagtggagaaatacgactctctggctgcttagattatgagaccgctcctcagtttacactgctaatcagagccagggactgtggagaaccgtcactgtcatccacgaccaccgttcacgtggatgtgcaagaaggcaacaaccacaggcctgcatttacccaggagaactataaggttcagattcctgaaggccgagccagccagggcgtgttgcgtctcctggttcaagatcgagattctccatttacatcagcttggagagcaaaattcaacatattgcatggcaatgaagaggggcattttgacatttcgactgaccctgagaccaacgaagggatattaaatgttatcaagcctttggattatgagactcgcccagcgcaaagcctcatcattgtcgtggagaatgaggagaggctcgtcttctgtgagagaggaaagcttcagccgccaaggaaggcagcagccagcgccactgtgagtgtgcaggtgacagacgccaacgacccaccagcctttcacccccagagcttcattgtcaataaagaggagggcgccaggcctgggaccctgttgggaacttttaatgccatggatccagacagccagataagatatgaactggttcatgacccagcaaattgggtcagcgtcgacaaaaactccggagtggtcatcaccgtggagccaattgaccgagaatcccctcatgtaaataacagtttttatgtaatcatcattcacgctgttgatgatggcttcccaccgcagactgctacagggaccctaatgctcttcctgtctgacatcaatgacaacgtcccgactctccggccacgttcccgctacatggaggtctgtgagtctgctgtgcatgagcccctccacatcgaggcagaggatccggacctggagccgttctctgacccatttacatttgaattggacaatacctggggaaatgcggaggacacatggaagttggggagaaattggggtcaatcagttgaacttttaaccttgagaagcctgccacgtggtaattacttggtgccactcttcattggagacaaacagggactttcccagaagcaaactgtccatgtaaggatctgcccctgtgccagtgggctcacatgtgtggagcttgcagatgcagaagtggggcttcatgtgggggccctgttccctgtctgtgcagcatttgtggctctggcagtggctctgctttttctgttgcgatgctattttgtgcttgaacctaagaggcatggatgctctgtatccaatgatgaaggccaccaaacactggtcatgtataatgcggagagcaaaggcacttcagcccagacatggtcagatgttgaaggccagaggccggctctgctcatctgcacagctgcagcaggacccacgcagggagttaaggatctcgaggaagtgcctccatctgcagcgagtcagtcagcccaagcacgctgtgctctggggagctggggttatggcaagccctttgagccaagaagtgtgaaaaacatacactctactcctgcttacccagatgccacaatgcacagacaactcctggctccggtggaaggaaggatggcagagacattgaatcagaaactccatgttgccaatgtgctggaagatgaccccggctacctacctcacgtctacagcgaggaaggggagtgtggaggggccccatccctcagctctctggccagcttggaacaggagttgcaacctgatttgctggactctttgggttcaaaagcgactccgtttgaggaaatatattcagagtcaggtgttccttcctaaaaaaaaaagtctattttggagaattgaaataattcatggaagggaatcactattcagggatttttcccctttgctcttcttttccctccttaaaagaaaaattaccttctagtcctaggatgaggacacactattagtttgaattaaatgctttgatattctcagatcagccatcttgaaccaaagcaaaaccacaagttacactttcttaaaatttgatttgtcatattttctagagaaacttgaatttaattgtgttattcttagcttccactggcagcctagctttgagggtaaatgaaaatataacccatagattacccagccacttgggaacagcaggtaatactgaagaaaaataaaaatagattttgaaaacgttacttacatttctatgattatgattctgcttccatttaagggaaaacttaggtaaatagagaaattttttctataacatttgtagtcagtatttgaagtgattttttaaaaaataagtattggtccctgttcactttttgattagataaatagataaaatatgttatcttgagaaaaatgattatgctgaaagctttataaacagtatactctttaaaaaatgaagagctgacataatttaacttgtatgtattatgtaagtaaaagagttaggagcctttgaatgagtaagttctgattagattttatctttaaacaaaaccacaaaatttaattggtttttacttgtccacttactgctagtgtcagtttcaggggaagaaatggtttcttttaaaaatcttaataggggacatatgccctaaaaatagtcagttttctagtctgagtaatagataagagactgactaagcaaagtttaaaatgctatttggacactttaatgcacatattggatatctaaaagtctacagccatataaaaattttatataattaatgagcaaatgccgtctctcatgccctaaaataaatcagtagaaacatgtttgctggtgaatcagtgaagcattatgttaaacagtgagttacagctcagagttaaaactttctccttctttttgaagaagctgtgcaaatacttctttttaaggagatctggccttttcctacctggttacctcagtcttcctctgctttgggaagctgaaaaagaagaaaaatcacatttaaagcactggaatgtctgaatgggacgcttgaatgtgtagaacagctgtactgatcctagcatgactcagaggacagtctagggcattttctgggtaattcaggataaaagtatttttttttttaagaaaaatacatgtttttggacaacaaaacaaagtaaacattagtttattcgattgcctccttatacttgcctctttcattctgtcccctgtagatttttaaaaaattatctcattttaaaactttattatttcattttaaataattgacatataataattgtacatatttagggggtacatagtcatgtttcaatacatttacagtgatcagatcagggtggttaacgtaatcattggctcaaacatttttcatttctttgtattggtacggagcattcaatatccatcccccttctagctatctaaaactatgtattattgttaactataggcaacatataatggtatagagtgctagaacgtattcctcctaggaataatttgctgtaattttgtatcctttaataaatctctccctatccctctttccccccacccttcccagctgctgtgtcctctgttctaccttctacttccgagataaacttggttttagcttcca

SEQ ID NO: 2 - DNA, 5391 bp, Homo sapiens
  source 1..5391: mol_type = other DNA; note = KCNJ2 cDNA ENST00000243457.4
agagcgcactggagccctggccagcgcgcagccttcccggcgccggcgggctgggtcttgggaattctggtttgctttggctcactcgctttttacaaaccactggatcttacatgcctctgtaccccccacttccactccatgtccccatgctcctgcgccagcaacaggacatgttctctggatgtcagctgagtcattaaagtaactctgcatgtcagtagacagaccttggtagaaccacaaggctcccagagacacccatctctcctcatttttttggtgtgtgtgtcttcaccgaacattcaaaactgtttctccaaagcgttttgcaaaaactcagactgttttccaaagcagaagcactggagtccccagcagaagcgatgggcagtgtgcgaaccaaccgctacagcatcgtctcttcagaagaagacggtatgaagttggccaccatggcagttgcaaatggctttgggaacgggaagagtaaagtccacacccgacaacagtgcaggagccgctttgtgaagaaagatggccactgtaatgttcagttcatcaatgtgggtgagaaggggcaacggtacctcgcagacatcttcaccacgtgtgtggacattcgctggcggtggatgctggttatcttctgcctggctttcgtcctgtcatggctgttttttggctgtgtgttttggttgatagctctgctccatggggacctggatgcatccaaagagggcaaagcttgtgtgtccgaggtcaacagcttcacggctgccttcctcttctccattgagacccagacaaccataggctatggtttcagatgtgtcacggatgaatgcccaattgctgttttcatggtggtgttccagtcaatcgtgggctgcatcatcgatgctttcatcattggcgcagtcatggccaagatggcaaagccaaagaagagaaacgagactcttgtcttcagtcacaatgccgtgattgccatgagagacggcaagctgtgtttgatgtggcgagtgggcaatcttcggaaaagccacttggtggaagctcatgttcgagcacagctcctcaaatccagaattacttctgaaggggagtatatccctctggatcaaatagacatcaatgttgggtttgacagtggaatcgatcgtatatttctggtgtccccaatcactatagtccatgaaatagatgaagacagtcctttatatgatttgagtaaacaggacattgacaacgcagactttgaaatcgtggtcatactggaaggcatggtggaagccactgccatgacgacacagtgccgtagctcttatctagcaaatgaaatcctgtggggccaccgctatgagcctgtgctctttgaagagaagcactactacaaagtggactattccaggttccacaaaacttacgaagtccccaacactcccctttgtagtgccagagacttagcagaaaagaaatatatcctctcaaatgcaaattcattttgctatgaaaatgaagttgccctcacaagcaaagaggaagacgacagtgaaaatggagttccagaaagcactagtacggacacgccccctgacatagaccttcacaaccaggcaagtgtacctctagagcccaggcccttacggcgagagtcggagatatgactgactgattccttctctggaatagttactttacaacacggtctgttggtcagaggcccaaaacagttatacagatgacggtactggtcaagatgggtcaagcaagcggccacaagggactgaggcaagcacaatggtttcaaagaaagactgtaagctccatgattagcataaagcactaaccatgtctccatgtgacccgatggcacatagatgttgtagaataagttatgggtttttatgttttgttttgtgtttttccaaaacttgaacttgcaggcaagccttggttgggtatttgatttatccagaatgcttctctttagggaacaaggatgtttttaatggcataacaaaggcaagactctgccttaatttttgaaaagctgctaactacatgaacacaaatgtgtatttttgttgcagtgtagttttccttttgtgtaattttaaagtcagtgttgaattttattgaaagctcatgatgcgcttcaaagtggcaagtatttggctattaactgccaaaacaagagcctgattttttgaggccagtaattcgtttgctagaattgattttttttctctctctctttgttacataagggcattatgtaacactagccgaatggtagcctctgggttgttgtttttttcttttcctccatgatgttaatgggttatctcaaattttaagttaaactacctaaaataaataccaaagataatgcatatttttgcacagtggagcttacacttaaaagaaaacaaagccccatgggctgccttgaaatcaagagacaataactttgaacctcagcaagaccttgaaccgccggttcattttgcaccttattcagaaaatagagcatcatactcaccgagtctagtcagtgtagtgcttttaaaaattttgtcctttcatgtaacttttttattttaagaggaagaagaagaaaggggcacacacacacaataccgacgtctatcctttcctgctaggcagtgctggccaggctcatgtgtagtgtgcgagatggtgatgtactcttatatttttctgggcttttccttttgcacattccaaaattcatttcataagacaagatcttcataggacctccttggcatcctggcattctcaaaactgagccatccagcatgaaagataaatgggtttaaacccttgctgctgaatttattgcctggactgtcaggacatcaccagcccaccttcaccttagggaagatgccacacctggcctccacacttgctcttctgatcagtctgtctggattgagtcctacagtgtcagatagggcggcaaatgccaaagcagggaaacagggaggtgtggacaagccagtttgatgcagcacttcagatcaagtgcttaggaaggagaggaaacttgccttttttatggcagaggatagtaatgaaaatgtctcagtattttagggtcaatgagagccataaaaatataacataatcacaagtaaaggagataatggtctaaaacagctatttcccttttctgtgtgcatacttatgactgaatgtgagctaagcattttctcctgtggagccctagagcaggttactaaggaaggacacattgttttccagaagcctcccctgcctggctgactgccttgctagaaacataattttttttttctcactgaagctcaataatggaactctttttttttttttttttaatttaaagttccctatttgtgaattctgggattactgacttttctttttaattggagtctcaaaatcaactctcttatggtattatatctctgtatgccattaaaaaacagcttgttctagaatcatgtattttgtaaactgatgtttgtgatggtctctggttcttgaacagccatatctgaatgccgtgcctgcaaaactatgacaatttttgctgttttcagccttcagatttgatggcttgggaaactgaggtgttattttcaatgaaacaaagaaagagatgttaagcaagtggttgttttagatccaaatgtaaaggcaggtttgggaaggtgtttaaagagttggaggaattggggattgagttgtaaagaaaacttacagaagaggcaacaatttggttcttgacagtgagaggatattgagggcttcagctgctgctattatgatgttttgcaaaggaaaataatcaaaccaaagagtattcagtgatatgtaaattaaatgaagatacagtggagaatgggggtgaccacaaaagaggctccccctaaacacacagtgctgccacttaaaaagacttgagaaatttgaaagggggtgggtatggggggggcaagaaagagggagggaaatctttcaacttatttctgaaaaagagaaaaaaatataaaatttctggtgcacaggtttgttttttcaagaaaattttgcagaagctatgtttttaaagtgtacattttataaagtttatcagatattttcatatttaaagccaaatgtaaatagaggtctgtaaagaaaaataattgccatagaaagtataatttcagtgcagtaatttctgagagctagtacctatatgctaccggttagcatggttttagcaaatatataccagccttataaggttcgtattgctatgttcttctgttatttatttcagcatggactgttcatttgaaacctttttctagttattagcgttttaacagttacaagctttaaatggcaattttttttttttttttttttttttttttttttttgtcaagagccaagacacaggtaatgcacgacattgattgctgcattttaccttcaaaatatttgtccttattgactgggtctccttaattaatgtacacatgtcattagaatgcagacggaggggactcaccatgaatatctggggttgattcccagatgtgtgttgcttctctattgcaagcagattccctgttggatttacttcggatttattcccttttaaagaatttttgcccatatctggaagggcactatatttttgggaggagccatagattcctggttatcctatttttaaacaaaatgtagacaaagtgaactctattttgattattgagaaaggagtagttttctatccctctaagagtatacttgaatcagacattttaaggatgtcactatggcactgttgtcatttccaaattcctagaaaagtttgttttactttgtttttattctgttaatgcattctttcttctctttacttcctttcttaccagtacactcctatctcaactctgtttatttgatgagttctgtcccgtaaatcatatttcccttacaattaataaatgtcacttcatattttataataaaccactcagtaaaagcaaaagcttgtcctgagaagtagagtgagttctttttcactctgtgtctaataatgttaaggtgggaaaaaaaaaagtgtggcatagctacctgcccatccccaaccctcagcaaagtagaatctcttttctggtaattttgggtttccgctctgggctctggcaagttgaacaatcctagccattgacaatcgtgatagttattattttcccatttgctgtctttttgtatctaaagtcttcctattgtactgcacaaaccatggattgtacatatttttatatattatgtcttattttattatttctaaataaaaaaattaaaaattgaaaa

SEQ ID NO: 3 - DNA, 6015 bp, Homo sapiens
  source 1..6015: mol_type = other DNA; note = PLD1 cDNA ENST00000351298.9
gctgagctccagctgtgccagaggcacccgagccctgagagtccgccgccaacgcgcaggtgctagcggccccttcgccctgcagcccctttgcttttactctgtccaaagttaacatgtcactgaaaaacgagccacgggtaaatacctctgcactgcagaaaattgctgctgacatgagtaatatcatagaaaatctggacacgcgggaactccactttgagggagaggaggtagactacgacgtgtctcccagcgatcccaagatacaagaagtgtatatccctttctctgctatttataacactcaaggatttaaggagcctaatatacagacgtatctctccggctgtccaataaaagcacaagttctggaagtggaacgcttcacatctacaacaagggtaccaagtattaatctttacactattgaattaacacatggggaatttaaatggcaagttaagaggaaattcaagcattttcaagaatttcacagagagctgctcaagtacaaagcctttatccgcatccccattcccactagaagacacacgtttaggaggcaaaacgtcagagaggagcctcgagagatgcccagtttgccccgttcatctgaaaacatgataagagaagaacaattccttggtagaagaaaacaactggaagattacttgacaaagatactaaaaatgcccatgtatagaaactatcatgccacaacagagtttcttgatataagccagctgtctttcatccatgatttgggaccaaagggcatagaaggtatgataatgaaaagatctggaggacacagaataccaggcttgaattgctgtggtcagggaagagcctgctacagatggtcaaaaagatggttaatagtgaaagattcctttttattgtatatgaaaccagacagcggtgccattgccttcgtcctgctggtagacaaagaattcaaaattaaggtggggaagaaggagacagaaacgaaatatggaatccgaattgataatctttcaaggacacttattttaaaatgcaacagctatagacatgctcggtggtggggaggggctatagaagaattcatccagaaacatggcaccaactttctcaaagatcatcgatttgggtcatatgctgctatccaagagaatgctttagctaaatggtatgttaatgccaaaggatattttgaagatgtggcaaatgcaatggaagaggcaaatgaagagatttttatcacagactggtggctgagtccagaaatcttcctgaaacgcccagtggttgagggaaatcgttggaggttggactgcattcttaaacgaaaagcacaacaaggagtgaggatcttcataatgctctacaaagaggtggaactcgctcttggcatcaatagtgaatacaccaagaggactttgatgcgtctacatcccaacataaaggtgatgagacacccggatcatgtgtcatccaccgtctatttgtgggctcaccatgagaagcttgtcatcattgaccaatcggtggcctttgtgggagggattgacctggcctatggaaggtgggacgacaatgagcacagactcacagacgtgggcagtgtgaagcgggtcacttcaggaccgtctctgggttccctcccacctgccgcaatggagtctatggaatccttaagactcaaagataaaaatgagcctgttcaaaacctacccatccagaagagtattgatgatgtggattcaaaactgaaaggaataggaaagccaagaaagttctccaaatttagtctctacaagcagctccacaggcaccacctgcacgacgcagatagcatcagcagcattgacagcacctccagttattttaatcactatagaagtcatcacaatttaatccatggtttaaaaccccacttcaaactctttcacccgtccagtgagtctgagcaaggactcactagacctcatgctgataccgggtccatccgtagtttacagacaggtgtgggagagctgcatggggaaaccagattctggcatggaaaggactactgcaatttcgtcttcaaagactgggttcaacttgataaaccttttgctgatttcattgacaggtactccacgccccggatgccctggcatgacattgcctctgcagtccacgggaaggcggctcgtgatgtggcacgtcacttcatccagcgctggaacttcacaaaaattatgaaatcaaaatatcggtccctttcttatccttttctgcttccaaagtctcaaacaacagcccatgagttgagatatcaagtgcctgggtctgtccatgctaacgtacagttgctccgctctgctgctgattggtctgctggtataaagtaccatgaagagtccatccacgccgcttacgtccatgtgatagagaacagcaggcactatatctatatcgaaaaccagtttttcataagctgtgctgatgacaaagttgtgttcaacaagataggcgatgccattgcccagaggatcctgaaagctcacagggaaaaccagaaataccgggtatatgtcgtgataccacttctgccagggttcgaaggagacatttcaaccggcggaggaaatgctctacaggcaatcatgcacttcaactacagaaccatgtgcagaggagaaaattccatccttggacagttaaaagcagagcttggtaatcagtggataaattacatatcattctgtggtcttagaacacatgcagagctcgaaggaaacctagtaactgagcttatctatgtccacagcaagttgttaattgctgatgataacactgttattattggctctgccaacataaatgaccgcagcatgctgggaaagcgtgacagtgaaatggctgtcattgtgcaagatacagagactgttccttcagtaatggatggaaaagagtaccaagctggccggtttgcccgaggacttcggctacagtgctttagggttgtccttggctatcttgatgacccaagtgaggacattcaggatccagtgagtgacaaattcttcaaggaggtgtgggtttcaacagcagctcgaaatgctacaatttatgacaaggttttccggtgccttcccaatgatgaagtacacaatttaattcagctgagagactttataaacaagcccgtattagctaaggaagatcccattcgagctgaggaggaactgaagaagatccgtggatttttggtgcaattccccttttatttcttgtctgaagaaagcctactgccttctgttgggaccaaagaggccatagtgcccatggaggtttggacttaagagatattcattggcagctcaaagacttccaccctggagaccacactgcacacagtgacttcctggggatgtcatagccaaagccaggcctgacgcattctcgtatccaacccaaggaccttttggaatgactggggagggctgcagtcacattgatgtaaggactgtaaacatcagcaagactttataattccttctgcctaacttgtaaaaagggggctgcattcttgttggtagcatgtactctgttgagtaaaacacatattcaaattccgtataccaaaatccatttcctttgtaacaagaatttaccagtaactgtgatctaggttgccaaaagttgtctgaatctccttattcttctctgatcttcatttatgcagccaatgtctagctggacctgccctcatcttgcagttcatacaggcactgtttgagagattgtttattattagatgttgtaatgctgcttcaagattcttcatggttacatgggatgcccctgctcatctggtcctgaagtagtaacattcacccaaatgaggatatagtcattattccttttcagtcactgtacgaacacggcagactttagcctacacagtagactgtgttaggcacttctggtaacattgacactgtatcttgacaccactaagcaacaggaaggaataaattccaatattgagacagagatttatttcattttgctcccaaaggcactgacaacatgagtccttgtgattaggcccacctgatcaaatgtaaaaacatgcatgggatatttgattacgtaacaaccagctaaaactgagagcacacagccttcggaaacccccaaggtgtcgaggaggatcagatccagataagagaagatgattccttctagtcctgtaaaatttcctgtcatccttagctgctgggttgattgaaatttgatctctacatttcaaaatcaaactagtgaatacagtttgtctttcaagagaatcagaggcatcgtaactcctaccaagttagtaagtatgagtctaaccttgtttgacattcaggtcttctgctacattatcttctttgagaaaaattaattgattataaaatatgtgctacttcacttacattattaaatatgtattaacgcctctcaccagggcttccagtgaagttacaatgccctagtctgtgaattagtctggaaacgtgtttttccttttcggatgttagagtaccctttgataaactaaattttactaagctgaacaactctgacagtctaaagagctaatgtgggttaccaaaaggcctgtacctgtaaaacaaaatgcaggtgtaatgattatacatgtctatggattacctggacatactctcatttgggttgttcttcaaagaagcaagcagccgatccctgttttcataaagctaatacttcagttggaaaaattaaacaggagcacaaagtcagggataggggttagcagaagagagaaatagtgtcacatcaagggcaggatctcatagctagggaacatttcacaaataaggtgagattttgtaaccaataataaaaatgaatgtttttataagtaaataacttatttttcatatggctaaagatggtaaaatgacttcattctatagccattgtaaataagaatttgctattgatgaaagaagttcagattggcatttgaagtattgagtgtatgggatctctaaggatttcttagattttatatttaaatattttttaaaccttagaggagtcaacaaactggctcttgattttcagcaccctactctcatgaaaaaagcctgaaaggaccctttcccttataagtaatttaatccaatttctccccattttatagatgaggaaactgaggctcagatcagatgagaactcacttaaatccactcaatgtgtagatggtagagctgggactagcaacattgctgcagcccattgttggcctctctcttcactttatcattgcccaagaatgaggatatgcagtaaacagaattcaggcaagatacctctaagctgttttgaaccctctgatattttgtatttatgtgtttgtctgtctccccctactagaatgtaagctccatggggcagggacttcactgtattttgttcatagtgtatccccagagcctggaccagtgcttggcacataggagatggcaataaatgcttgtagaattaataaacaaggtgaaggagagagctaatgaaatgaaaatcttagtctcatataagaagtcttactactgctttctatggcaagttccttttctattgcatcttcccaaagacaagatgctcatctgcaaaggggtgataagatttacttggagggattttatggaaaattcagtgcaataattgcttttttttttttttttgcagtagcagtttacatagtacagcattctgcaaaaattgcatgaaatgtggacacaagatgtactgtatgacttaattacctgtcattctctgacaccattactacctactagaagttcaaataatttatctttaacattgcaatatctgataaactttttaaaatgtaaataattcaaagccttgaaaatctatcatgaatctgctcaacatttcaaagtgactattttgaaatgcctataaatgctatatacctga

SEQ ID NO: 4 - DNA, 24 bp, synthetic construct
  source 1..24: mol_type = other DNA; note = CDH26 probe; note (original language) = sonda CDH26; organism (original language) = construccion sintetica
tacccagatgccacaatgcacaga

SEQ ID NO: 5 - DNA, 20 bp, synthetic construct
  source 1..20: mol_type = other DNA; note = CDH26 primer 1; note (original language) = cebador 1 CDH26; organism (original language) = construccion sintetica
gtctctgccatccttccttc

SEQ ID NO: 6 - DNA, 18 bp, synthetic construct
  source 1..18: mol_type = other DNA; note = CDH26 primer 2; note (original language) = cebador 2 CDH26; organism (original language) = construccion sintetica
gcaagccctttgagccaa

SEQ ID NO: 7 - DNA, 22 bp, synthetic construct
  source 1..22: mol_type = other DNA; note = KCNJ2 probe; note (original language) = sonda KCNJ2; organism (original language) = construccion sintetica
ccacttccactccatgtcccca

SEQ ID NO: 8 - DNA, 20 bp, synthetic construct
  source 1..20: mol_type = other DNA; note = KCNJ2 primer 1; note (original language) = cebador 1 KCNJ2; organism (original language) = construccion sintetica
cagctgacatccagagaaca

SEQ ID NO: 9 - DNA, 22 bp, synthetic construct
  source 1..22: mol_type = other DNA; note = KCNJ2 primer 2; note (original language) = cebador 2 KCNJ2; organism (original language) = construccion sintetica
gctcactcgctttttacaaacc

SEQ ID NO: 10 - DNA, 24 bp, synthetic construct
  source 1..24: mol_type = other DNA; note = PLD1 probe; note (original language) = sonda PLD1; organism (original language) = construccion sintetica
tgctgctgattggtctgctggtat

SEQ ID NO: 11 - DNA, 21 bp, synthetic construct
  source 1..21: mol_type = other DNA; note = PLD1 primer 1; note (original language) = cebador 1 PLD1; organism (original language) = construccion sintetica
gcctgctgttctctatcacat

SEQ ID NO: 12 - DNA, 21 bp, synthetic construct
  source 1..21: mol_type = other DNA; note = PLD1 primer 2; note (original language) = cebador 2 PLD1; organism (original language) = construccion sintetica
gtctgtccatgctaacgtaca

SEQ ID NO: 13 - DNA, 24 bp, synthetic construct
  source 1..24: mol_type = other DNA; note = CRYAB probe; note (original language) = sonda CRYAB; organism (original language) = construccion sintetica
agcacttctccccagaggaactca

SEQ ID NO: 14 - DNA, 21 bp, synthetic construct
  source 1..21: mol_type = other DNA; note = CRYAB primer 1; note (original language) = cebador 1 CRYAB; organism (original language) = construccion sintetica
caatcacatctcccaacacct

SEQ ID NO: 15 - DNA, 21 bp, synthetic construct
  source 1..21: mol_type = other DNA; note = CRYAB primer 2; note (original language) = cebador 2 CRYAB; organism (original language) = construccion sintetica
ctggtttgacactggactctc

SEQ ID NO: 16 - DNA, 22 bp, synthetic construct
  source 1..22: mol_type = other DNA; note = FAM43A probe; note (original language) = sonda FAM43A; organism (original language) = construccion sintetica
ttcccctctcaaatctccccgc

SEQ ID NO: 17 - DNA, 19 bp, synthetic construct
  source 1..19: mol_type = other DNA; note = FAM43A primer 1; note (original language) = cebador 1 FAM43A; organism (original language) = construccion sintetica
aacttcagccaaccttccc

SEQ ID NO: 18 - DNA, 19 bp, synthetic construct
  source 1..19: mol_type = other DNA; note = FAM43A primer 2; note (original language) = cebador 2 FAM43A; organism (original language) = construccion sintetica
cacttttggctctgttgcg

SEQ ID NO: 19 - DNA, 22 bp, synthetic construct
  source 1..22: mol_type = other DNA; note = SDR9C7 probe; note (original language) = sonda SDR9C7; organism (original language) = construccion sintetica
cccactttgtccctcacccact

SEQ ID NO: 20 - DNA, 19 bp, synthetic construct
  source 1..19: mol_type = other DNA; note = SDR9C7 primer 1; note (original language) = cebador 1 SDR9C7; organism (original language) = construccion sintetica
caccagcattgttcaccag

SEQ ID NO: 21 - DNA, 20 bp, synthetic construct
  source 1..20: mol_type = other DNA; note = SDR9C7 primer 2; note (original language) = cebador 2 SDR9C7; organism (original language) = construccion sintetica
ggatgtcaccaagagcgaaa

SEQ ID NO: 22 - DNA, 26 bp, synthetic construct
  source 1..26: mol_type = other DNA; note = LINC00707 probe; note (original language) = sonda LINC00707; organism (original language) = construccion sintetica
atgatcacaaggtgaggtcccacaac

SEQ ID NO: 23 - DNA, 21 bp, synthetic construct
  source 1..21: mol_type = other DNA; note = LINC00707 primer 1; note (original language) = cebador 1 LINC00707; organism (original language) = construccion sintetica
cagatgtgcaggaggtgttag

SEQ ID NO: 24 - DNA, 22 bp, synthetic construct
  source 1..22: mol_type = other DNA; note = LINC00707 primer 2; note (original language) = primer 2 LINC00707; organism (original language) = construccion sintetica
gactttactggctttcttgctc

SEQ ID NO: 25 - DNA, 24 bp, synthetic construct
  source 1..24: mol_type = other DNA; note = KCNJ2-AS1 probe; note (original language) = sonda KCNJ2-AS1; organism (original language) = construccion sintetica
cagatccgcacttactcctgcctt

SEQ ID NO: 26 - DNA, 22 bp, synthetic construct
  source 1..22: mol_type = other DNA; note = KCNJ2-AS1 primer 1; note (original language) = cebador 1 KCNJ2-AS1; organism (original language) = construccion sintetica
aagtaccttgctcagtgctaag

SEQ ID NO: 27 - DNA, 21 bp, synthetic construct
  source 1..21: mol_type = other DNA; note = KCNJ2-AS1 primer 2; note (original language) = cebador 2 KCNJ2-AS1; organism (original language) = construccion sintetica
ctcccatcctcatatccacac